European Patent Specification EP 3 578 193 B1, published September 6, 2023. Title: Compounds and their use. Applicant: NovaBiotics Limited. Application PCT/GB2011/000480. The sequence listing filed with the application follows.

SEQUENCE LISTING (26 sequences)

SEQ ID NO: 1 - protein, 13 aa, Artificial
  synthetic peptide
RRRFRFFFRFRRR

SEQ ID NO: 2 - protein, 13 aa, Artificial
  synthetic peptide
HHHFRFFFRFRRR

SEQ ID NO: 3 - protein, 14 aa, Artificial
  sythetic peptide
KKFPWRLRLRYGRR

SEQ ID NO: 4 - protein, 13 aa, Artificial
  synthetic peptide
RRRRRFFFRFRRR

SEQ ID NO: 5 - protein, 13 aa, Artificial
  synthetic peptide
RRRFRFRFRFRRR

SEQ ID NO: 6 - protein, 13 aa, Artificial
  synthetic peptide
RRRFRFPFRFRRR

SEQ ID NO: 7 - protein, 13 aa, Artificial
  synthetic peptide
RRFRRFFFRRFRR

SEQ ID NO: 8 - protein, 11 aa, Artificial
  synthetic peptide
RRRRFFFRRRR

SEQ ID NO: 9 - protein, 11 aa, Artificial
  synthetic peptide
RRRRFRFRRRR

SEQ ID NO: 10 - protein, 11 aa, Artificial
  synthetic peptide
RRRRFPFRRRR

SEQ ID NO: 11 - protein, 11 aa, Artificial
  synthetic peptide
RRFRRRFRRFR

SEQ ID NO: 12 - protein, 11 aa, Artificial
  synthetic peptide
RRFRRRFRRFG

SEQ ID NO: 13 - protein, 11 aa, Artificial
  synthetic peptide
RRFGRRFRRFG

SEQ ID NO: 14 - protein, 11 aa, Artificial
  synthetic peptide
RRFRRFRRRFG

SEQ ID NO: 15 - protein, 11 aa, Artificial
  synthetic peptide
RRFRRFRRRFR

SEQ ID NO: 16 - protein, 13 aa, Artificial
  synthetic peptide
FRRRRFFFRFRRR

SEQ ID NO: 17 - protein, 13 aa, Artificial
  syntheic peptide
RRRRRFFFRRRRF

SEQ ID NO: 18 - protein, 13 aa, Artificial
  synthetic peptide
FFFFRRRRRFRRR

SEQ ID NO: 19 - protein, 13 aa, Artificial
  synthetic peptide
RRRRFFFFFRRRR

SEQ ID NO: 20 - protein, 13 aa, Artificial
  synthetic peptide
FRRRRFFFRRRRF

SEQ ID NO: 21 - protein, 13 aa, Artificial
  synthetic peptide
RRRYRYYYRYRRR

SEQ ID NO: 22 - protein, 13 aa, Artificial
  synthetic peptide
RRRARAAARARRR

SEQ ID NO: 23 - protein, 13 aa, Artificial
  synthetic peptide
RRRFRRRRRFFFF

SEQ ID NO: 24 - protein, 13 aa, Artificial
  synthetic peptide
RRRFFFFFFFRRR

SEQ ID NO: 25 - protein, 13 aa, Artificial
  synthetic peptide
RRRFRFFFRFRRR

SEQ ID NO: 26 - protein, 14 aa, Artificial
  synthetic peptide
KKPRRKPRRPKRKK